European Patent Specification EP 3 371 204 B1, published May 8, 2024. Title: Genetically Modified Microorganisms. Applicant: University of Kent. Application GB1519554.8. The sequence listing filed with the application follows.

SEQUENCE LISTING (79 sequences)

SEQ ID NO: 1 - protein, 9 aa, Artificial Sequence
  Synthetic Sequence
LEQIIRDVL

SEQ ID NO: 2 - protein, 9 aa, Artificial Sequence
  Synthetic Sequence
LETLIRTIL

SEQ ID NO: 3 - protein, 9 aa, Artificial Sequence
  Synthetic Sequence
LETLIRNIL

SEQ ID NO: 4 - protein, 9 aa, Artificial Sequence
  Synthetic Sequence
LRQIIEDVL

SEQ ID NO: 5 - protein, 9 aa, Artificial Sequence
  Synthetic Sequence
IEEIVRSVM

SEQ ID NO: 6 - protein, 9 aa, Artificial Sequence
  Synthetic Sequence
IEQVVKAVL

SEQ ID NO: 7 - protein, 9 aa, Artificial Sequence
  Synthetic Sequence
VEKLVRQAI

SEQ ID NO: 8 - protein, 9 aa, Artificial Sequence
  Synthetic Sequence
IQEIVRTLI

SEQ ID NO: 9 - protein, 9 aa, Artificial Sequence
  Synthetic Sequence
VEEIVKRIM

SEQ ID NO: 10 - protein, 9 aa, Artificial Sequence
  Synthetic Sequence
IESMVRDVL

SEQ ID NO: 11 - protein, 9 aa, Artificial Sequence
  Synthetic Sequence
VQDIIKNVV

SEQ ID NO: 12 - protein, 9 aa, Artificial Sequence
  Synthetic Sequence
IRQVVQEVL

SEQ ID NO: 13 - protein, 9 aa, Artificial Sequence
  Synthetic Sequence
VRSVVEEVV

SEQ ID NO: 14 - protein, 9 aa, Artificial Sequence
  Synthetic Sequence
ARDLLKQIL

SEQ ID NO: 15 - protein, 18 aa, Artificial Sequence
  Synthetic Sequence
  VARIANT (1)..(1): /replace="Ile"
  VARIANT (2)..(2): /replace="Tyr"
  VARIANT (4)..(4): /replace="Lys"
  VARIANT (5)..(5): /replace="Ala" /replace="Gly" /replace="Glu"
  VARIANT (6)..(6): /replace="Ser" /replace="Gln"
  VARIANT (7)..(7): /replace="Val" /replace="Leu" /replace="Phe"
  VARIANT (8)..(8): /replace="Gln" /replace="Ser" /replace="Leu"
  VARIANT (9)..(9): /replace="Gln" /replace="Arg"
  VARIANT (10)..(10): /replace="Leu"
  VARIANT (11)..(11): /replace="Met" /replace="Arg"
  VARIANT (12)..(12): /replace="Leu" /replace="Cys" /replace="Gln"
  VARIANT (13)..(13): /replace="Ser"
  VARIANT (14)..(14): /replace="Met"
  VARIANT (17)..(17): /replace="Asp" /replace="Glu"
  VARIANT (18)..(18): /replace="Asn" /replace="Gln"
VVGQVYINKMLVTLFPHR

SEQ ID NO: 16 - protein, 13 aa, Artificial Sequence
  Synthetic Sequence
  VARIANT (1)..(1): /replace="Phe"
  VARIANT (2)..(2): /replace="Pro" /replace="Ala"
  VARIANT (3)..(3): /replace="Val"
  VARIANT (4)..(4): /replace="Gln"
  VARIANT (6)..(6): /replace="Ser" /replace="Gln" /replace="Trp"
  VARIANT (7)..(7): /replace="Glu" /replace="Arg"
  VARIANT (11)..(11): /replace="Gln"
  VARIANT (13)..(13): /replace="Asn"
LSPEQAQRIYRGS

SEQ ID NO: 17 - protein, 16 aa, Artificial Sequence
  Synthetic Sequence
  VARIANT (2)..(2): /replace="Asn"
  VARIANT (3)..(3): /replace="Gln"
  VARIANT (4)..(4): /replace="Gln"
  VARIANT (5)..(5): /replace="Glu"
  VARIANT (6)..(6): /replace="Ile"
  VARIANT (7)..(7): /replace="Arg" /replace="Glu"
  VARIANT (8)..(8): /replace="Asp"
  VARIANT (9)..(9): /replace="Met"
  VARIANT (10)..(10): /replace="Ile"
  VARIANT (11)..(11): /replace="Glu"
  VARIANT (12)..(12): /replace="Gln"
  VARIANT (13)..(13): /replace="Ile"
  VARIANT (14)..(14): /replace="Met"
  VARIANT (16)..(16): /replace="Gln" /replace="Ser"
MDEKQLKEIVRSVLAE

SEQ ID NO: 18 - protein, 16 aa, Artificial Sequence
  Synthetic Sequence
  VARIANT (1)..(1): /replace="Lys" /replace="Ser"
  VARIANT (2)..(2): /replace="Asp"
  VARIANT (3)..(3): /replace="Glu"
  VARIANT (5)..(5): /replace="Val"
  VARIANT (6)..(6): /replace="Asp" /replace="Asn"
  VARIANT (7)..(7): /replace="glu" /replace="Ser"
  VARIANT (8)..(8): /replace="Leu"
  VARIANT (9)..(9): /replace="Ile"
  VARIANT (10)..(10): /replace="Lys" /replace="Glu" /replace="Gln"
  VARIANT (11)..(11): /replace="Arg"
  VARIANT (14)..(14): /replace="Ala"
  VARIANT (15)..(15): /replace="Lys"
AEALIELIVRKVLEEL

SEQ ID NO: 19 - protein, 18 aa, Artificial Sequence
  Synthetic Sequence
  VARIANT (4)..(4): /replace="Asp" /replace="Thr"
  VARIANT (6)..(6): /replace="Glu"
  VARIANT (7)..(7): /replace="Val"
  VARIANT (8)..(8): /replace="Val"
  VARIANT (9)..(9): /replace="Glu"
  VARIANT (11)..(11): /replace="Val"
  VARIANT (12)..(12): /replace="Val"
  VARIANT (13)..(13): /replace="Lys" /replace="Ala"
  VARIANT (14)..(14): /replace="Glu"
  VARIANT (17)..(17): /replace="Ser" /replace="Arg" /replace="Ala"
  VARIANT (18)..(18): /replace="Asp"
MEINEKLLRQIIEDVLKE

SEQ ID NO: 20 - protein, 18 aa, Artificial Sequence
  Synthetic Sequence
  VARIANT (1)..(1): /replace="Ile"
  VARIANT (2)..(2): /replace="Asp"
  VARIANT (3)..(3): /replace="Glu"
  VARIANT (4)..(4): /replace="Lys"
  VARIANT (5)..(5): /replace="Leu"
  VARIANT (6)..(6): /replace="Leu"
  VARIANT (8)..(8): /replace="Glu"
  VARIANT (9)..(9): /replace="Ile"
  VARIANT (11)..(11): /replace="Lys"
  VARIANT (12)..(12): /replace="Glu" /replace="Gln"
  VARIANT (15)..(15): /replace="Asn"
  VARIANT (16)..(16): /replace="Leu"
  VARIANT (17)..(17): /replace="Glu" /replace="Gly"
MNTDAIESMVRDVLSMNS

SEQ ID NO: 21 - protein, 16 aa, Artificial Sequence
  Synthetic Sequence
  VARIANT (2)..(2): /replace="Asp" /replace="Glu"
  VARIANT (3)..(3): /replace="Ser" /replace="Glu"
  VARIANT (4)..(4): /replace="Leu"
  VARIANT (6)..(6): /replace="Val"
  VARIANT (8)..(8): /replace="Gln" /replace="Lys" /replace="Asp"
  VARIANT (9)..(9): /replace="Ile"
  VARIANT (10)..(10): /replace="Val"
  VARIANT (11)..(11): /replace="Lys"
  VARIANT (12)..(12): /replace="Asn" /replace="Lys"
  VARIANT (13)..(13): /replace="Val"
  VARIANT (14)..(14): /replace="Ile"
  VARIANT (15)..(15): /replace="Leu" /replace="Arg" /replace="Asn"
MNTSELETLIRTILSE

SEQ ID NO: 22 - protein, 26 aa, Artificial Sequence
  Synthetic Sequence
  VARIANT (1)..(1): /replace="Pro"
  VARIANT (2)..(2): /replace="Gly"
  VARIANT (3)..(3): /replace="Gln"
  VARIANT (4)..(4): /replace="Asp"
  VARIANT (5)..(5): /replace="Ala"
  VARIANT (6)..(6): /replace="Asn"
  VARIANT (8)..(8): /replace="Gln"
  VARIANT (9)..(9): /replace="Gln"
  VARIANT (10)..(10): /replace="Val"
  VARIANT (12)..(12): /replace="Glu"
  VARIANT (16)..(16): /replace="Arg"
  VARIANT (17)..(17): /replace="Ile"
  VARIANT (18)..(18): /replace="Ile"
  VARIANT (19)..(19): /replace="Gly"
  VARIANT (20)..(20): /replace="Glu" /replace="Ser"
  VARIANT (21)..(21): /replace="Ser"
  VARIANT (23)..(23): /replace="Ser"
  VARIANT (26)..(26): /replace="Val"
AKSSLTEEDIYDAVKKVLEQHGALDP

SEQ ID NO: 23 - protein, 19 aa, Artificial Sequence
  Synthetic Sequence
  VARIANT (3)..(3): /replace="Thr"
  VARIANT (4)..(4): /replace="Thr"
  VARIANT (5)..(5): /replace="Gln"
  VARIANT (6)..(6): /replace="Leu"
  VARIANT (7)..(7): /replace="Glu"
  VARIANT (8)..(8): /replace="Asn"
  VARIANT (9)..(9): /replace="Met"
  VARIANT (10)..(10): /replace="Ile"
  VARIANT (11)..(11): /replace="Arg" /replace="Ala"
  VARIANT (12)..(12): /replace="Lys" /replace="Asn"
  VARIANT (15)..(15): /replace="Ala" /replace="Glu" /replace="Arg"
  VARIANT (16)..(16): /replace="Lys"
  VARIANT (17)..(17): /replace="Phe" /replace="Tyr"
  VARIANT (18)..(18): /replace="Leu" /replace="Gly"
MNDIEIAQAVSTILSDNTK

SEQ ID NO: 24 - protein, 21 aa, Artificial Sequence
  Synthetic Sequence
  VARIANT (3)..(3): /replace="Glu"
  VARIANT (6)..(6): /replace="Val"
  VARIANT (7)..(7): /replace="Gly"
  VARIANT (9)..(9): /replace="Ile"
  VARIANT (10)..(10): /replace="Ala"
  VARIANT (12)..(12): /replace="Gln"
  VARIANT (14)..(14): /replace="Leu"
  VARIANT (16)..(16): /replace="Gly"
  VARIANT (17)..(17): /replace="Met"
  VARIANT (18)..(18): /replace="Gln"
  VARIANT (19)..(19): /replace="Asp"
LDAESAADMTEMIAKELKEAG

SEQ ID NO: 25 - protein, 18 aa, Artificial Sequence
  Synthetic Sequence
  VARIANT (1)..(1): /replace="Pro"
  VARIANT (2)..(2): /replace="Asn"
  VARIANT (3)..(3): /replace="Glu"
  VARIANT (4)..(4): /replace="Glu" /replace="Ala"
  VARIANT (6)..(6): /replace="Ile"
  VARIANT (8)..(8): /replace="Ala" /replace="Ser"
  VARIANT (11)..(11): /replace="Arg"
  VARIANT (12)..(12): /replace="Arg" /replace="Gln"
  VARIANT (14)..(14): /replace="Leu"
  VARIANT (15)..(15): /replace="Glu"
  VARIANT (18)..(18): /replace="Lys"
DDADLVAEITKKVMAQLG

SEQ ID NO: 26 - protein, 20 aa, Artificial Sequence
  Synthetic Sequence
  VARIANT (5)..(5): /replace="Met"
  VARIANT (11)..(11): /replace="Arg" /replace="Lys"
  VARIANT (16)..(16): /replace="Arg"
  VARIANT (20)..(20): /replace="Thr"
VNEQLVQDIVQEVVAKMQIS

SEQ ID NO: 27 - protein, 19 aa, Artificial Sequence
  Synthetic Sequence
  VARIANT (4)..(4): /replace="Gln"
  VARIANT (7)..(7): /replace="Gln"
  VARIANT (8)..(8): /replace="Leu"
  VARIANT (11)..(11): /replace="Glu"
  VARIANT (12)..(12): /replace="Arg" /replace="Glu"
  VARIANT (16)..(16): /replace="Glu"
  VARIANT (18)..(18): /replace="Ser"
DQEALVKAITDQVMAALKK

SEQ ID NO: 28 - protein, 20 aa, Artificial Sequence
  Artificial Sequence
  VARIANT (3)..(3): /replace="Ala"
  VARIANT (4)..(4): /replace="Thr"
  VARIANT (7)..(7): /replace="Thr"
  VARIANT (13)..(13): /replace="Gln"
  VARIANT (14)..(14): /replace="Glu"
  VARIANT (17)..(17): /replace="Ser"
  VARIANT (18)..(18): /replace="Gln"
  VARIANT (19)..(19): /replace="Leu"
  VARIANT (20)..(20): /replace="Asn"
MQIDEELIRSVVAQVLAEVG

SEQ ID NO: 29 - protein, 15 aa, Artificial Sequence
  Synthetic Sequence
  VARIANT (1)..(1): /replace="Gln" /replace="Asp"
  VARIANT (2)..(2): /replace="Glu" /replace="Asp"
  VARIANT (3)..(3): /replace="Ile" /replace="Leu"
  VARIANT (4)..(4): /replace="Gln" /replace="Ala"
  VARIANT (5)..(5): /replace="Gln" /replace="Asp"
  VARIANT (6)..(6): /replace="Leu" /replace="Val"
  VARIANT (7)..(7): /replace="Leu" /replace="Val"
  VARIANT (8)..(8): /replace="Arg" /replace="Asn"
  VARIANT (9)..(9): /replace="Gln" /replace="Lys"
  VARIANT (10)..(10): /replace="Ile" /replace="Leu"
  VARIANT (11)..(11): /replace="Ile" /replace="Val"
  VARIANT (12)..(12): /replace="Gln" /replace="Gly"
  VARIANT (13)..(13): /replace="Arg" /replace="Ala"
  VARIANT (14)..(14): /replace="Met"
  VARIANT (15)..(15): /replace="Gly" /replace="Ser"
ENVERIIKEVLEQLK

SEQ ID NO: 30 - protein, 16 aa, Artificial Sequence
  Synthetic Sequence
  VARIANT (2)..(2): /replace="Asp"
  VARIANT (3)..(3): /replace="Ile" /replace="Asn" /replace="Leu"
  VARIANT (4)..(4): /replace="Tyr"
  VARIANT (5)..(5): /replace="Asn" /replace="Ser" /replace="Leu" /replace="Phe"
  VARIANT (6)..(6): /replace="Ser"
  VARIANT (7)..(7): /replace="Asn"
  VARIANT (8)..(8): /replace="Lys"
  VARIANT (9)..(9): /replace="Leu" /replace="Phe"
  VARIANT (10)..(10): /replace="Ala"
  VARIANT (11)..(11): /replace="Val" /replace="Met"
  VARIANT (12)..(12): /replace="Ala"
  VARIANT (13)..(13): /replace="Thr"
  VARIANT (14)..(14): /replace="Lys"
  VARIANT (15)..(15): /replace="Asn"
  VARIANT (16)..(16): /replace="Met"
MAKRETPRVKELAERL

SEQ ID NO: 31 - protein, 22 aa, Artificial Sequence
  Synthetic Sequence
  VARIANT (2)..(2): /replace="Asp" /replace="Gly"
  VARIANT (5)..(5): /replace="Gle" /replace="Asp"
  VARIANT (10)..(10): /replace="Arg"
  VARIANT (12)..(12): /replace="Ile"
  VARIANT (13)..(13): /replace="Ala"
  VARIANT (17)..(17): /replace="Arg"
  VARIANT (18)..(18): /replace="Glu"
  VARIANT (20)..(20): /replace="Asn" /replace="Gly"
  VARIANT (21)..(21): /replace="Arg"
  VARIANT (22)..(22): /replace="Gln"
IEALRAELRALVVEELAQLIKR

SEQ ID NO: 32 - protein, 18 aa, Artificial Sequence
  Synthetic Sequence
  VARIANT (1)..(1): /replace="Ile"
  VARIANT (2)..(2): /replace="Tyr"
  VARIANT (4)..(4): /replace="Lys"
  VARIANT (5)..(5): /replace="Ala" /replace="Gly" /replace="Glu"
  VARIANT (6)..(6): /replace="Ser" /replace="Gln"
  VARIANT (7)..(7): /replace="Val" /replace="Leu" /replace="Phe"
  VARIANT (8)..(8): /replace="Gln" /replace="Ser"
  VARIANT (9)..(9): /replace="Gln" /replace="Arg"
  VARIANT (10)..(10): /replace="Leu"
  VARIANT (11)..(11): /replace="Met"
  VARIANT (12)..(12): /replace="Gln"
  VARIANT (13)..(13): /replace="Ser"
  VARIANT (14)..(14): /replace="Met"
  VARIANT (17)..(17): /replace="Asp" /replace="Glu"
  VARIANT (18)..(18): /replace="Asn" /replace="Gln"
VVGQVYINKMLCTLFPHR

SEQ ID NO: 33 - protein, 16 aa, Artificial Sequence
  Synthetic Sequence
  VARIANT (1)..(1): /replace="Lys" /replace="Ser"
  VARIANT (2)..(2): /replace="Asp"
  VARIANT (3)..(3): /replace="Glu"
  VARIANT (5)..(5): /replace="Val"
  VARIANT (6)..(6): /replace="Asp" /replace="Asn"
  VARIANT (7)..(7): /replace="Ser"
  VARIANT (8)..(8): /replace="Leu"
  VARIANT (9)..(9): /replace="Ile"
  VARIANT (10)..(10): /replace="Lys" /replace="Glu" /replace="Gln"
  VARIANT (11)..(11): /replace="Arg"
  VARIANT (14)..(14): /replace="Ala"
  VARIANT (15)..(15): /replace="Lys"
AEALIEEIVRKVLEEL

SEQ ID NO: 34 - protein, 19 aa, Artificial Sequence
  Synthetic Sequence
  VARIANT (3)..(3): /replace="Asp" /replace="Thr"
  VARIANT (6)..(6): /replace="Glu"
  VARIANT (7)..(7): /replace="Val"
  VARIANT (8)..(8): /replace="Val"
  VARIANT (9)..(9): /replace="Glu"
  VARIANT (11)..(11): /replace="Val"
  VARIANT (12)..(12): /replace="Val"
  VARIANT (13)..(13): /replace="Lys"
  VARIANT (14)..(14): /replace="Glu"
  VARIANT (17)..(17): /replace="Ser" /replace="Arg" /replace="Ala"
  VARIANT (18)..(18): /replace="Asp"
  VARIANT (19)..(19): /replace="Leu"
MEINEKLLRQIIEDVLKEM

SEQ ID NO: 35 - protein, 19 aa, Artificial Sequence
  Synthetic Sequence
  VARIANT (3)..(3): /replace="Thr"
  VARIANT (4)..(4): /replace="Thr"
  VARIANT (5)..(5): /replace="Gln"
  VARIANT (6)..(6): /replace="Leu"
  VARIANT (8)..(8): /replace="Asn"
  VARIANT (9)..(9): /replace="Met"
  VARIANT (10)..(10): /replace="Ile"
  VARIANT (11)..(11): /replace="Arg"
  VARIANT (12)..(12): /replace="Lys" /replace="Asn"
  VARIANT (15)..(15): /replace="Ala" /replace="Glu" /replace="Arg"
  VARIANT (16)..(16): /replace="Lys"
  VARIANT (17)..(17): /replace="Phe" /replace="Tyr"
  VARIANT (18)..(18): /replace="Leu" /replace="Gly"
MNDIEIEQAVSTILSDNTK

SEQ ID NO: 36 - protein, 20 aa, Artificial Sequence
  Synthetic Sequence
  VARIANT (3)..(3): /replace="Ala"
  VARIANT (4)..(4): /replace="Thr"
  VARIANT (7)..(7): /replace="Thr"
  VARIANT (14)..(14): /replace="Glu"
  VARIANT (17)..(17): /replace="Ser"
  VARIANT (18)..(18): /replace="Gln"
  VARIANT (19)..(19): /replace="Leu"
  VARIANT (20)..(20): /replace="Asn"
MQIDEELIRSVVQQVLAEVG

SEQ ID NO: 37 - protein, 15 aa, Artificial Sequence
  Synthetic Sequence
  VARIANT (1)..(1): /replace="Gln" /replace="Asp"
  VARIANT (2)..(2): /replace="Glu" /replace="Asp"
  VARIANT (3)..(3): /replace="Ile" /replace="Leu"
  VARIANT (4)..(4): /replace="Gln"
  VARIANT (5)..(5): /replace="Gln" /replace="Asp"
  VARIANT (6)..(6): /replace="Leu" /replace="Val"
  VARIANT (7)..(7): /replace="Leu" /replace="Val"
  VARIANT (8)..(8): /replace="Arg" /replace="Asn"
  VARIANT (9)..(9): /replace="Gln" /replace="Lys"
  VARIANT (10)..(10): /replace="Ile" /replace="Leu"
  VARIANT (11)..(11): /replace="Ile" /replace="Val"
  VARIANT (12)..(12): /replace="Gln" /replace="Gly"
  VARIANT (13)..(13): /replace="Arg" /replace="Ala"
  VARIANT (14)..(14): /replace="Met"
  VARIANT (15)..(15): /replace="Gly" /replace="Ser"
ENVERIIKEVLEQLK

SEQ ID NO: 38 - protein, 18 aa, Synechococcus elongatus
VYGKEQFLRMRQSMFPDR

SEQ ID NO: 39 - protein, 13 aa, Synechococcus elongatus
LAPEQQQRIYRGN

SEQ ID NO: 40 - protein, 16 aa, Salmonella typhimurium
MDQKQIEEIVRSVMAS

SEQ ID NO: 41 - protein, 17 aa, Clostridium phytofermentans
MNQQDIEQVVKAVLLKM

SEQ ID NO: 42 - protein, 16 aa, Clostridium phytofermentans
NTELVEEIVKRIMKQL

SEQ ID NO: 43 - protein, 19 aa, Salmonella typhimurium
MEINEKLLRQIIEDVLRDM

SEQ ID NO: 44 - protein, 18 aa, Salmonella typhimurium
MEINEKLLRQIIEDVLRD

SEQ ID NO: 45 - protein, 18 aa, Artificial Sequence
  Synthetic Sequence
MEINEKLLRQIIEDVLSE

SEQ ID NO: 46 - protein, 19 aa, Salmonella typhimurium
MNTDAIESMVRDVLSRMNS

SEQ ID NO: 47 - protein, 16 aa, Salmonella typhimurium
MNTSELETLIRTILSE

SEQ ID NO: 48 - protein, 16 aa, Artificial Sequence
  Synthetic Sequence
MNTSELETLIRNILSE

SEQ ID NO: 49 - protein, 18 aa, Artificial Sequence
  Synthetic Sequence
MNTSELETLIRNILSEQL

SEQ ID NO: 50 - protein, 26 aa, Rhodopseudomonas palustris
AGTNYTEEQVFAAVKKVLNSSGSTDV

SEQ ID NO: 51 - protein, 19 aa, Rhodopseudomonas palustris
MVAKAIRDHAGTAQPSGNA

SEQ ID NO: 52 - protein, 21 aa, Clostridium phytofermentans
IDIILAQQITVQIVKELKERG

SEQ ID NO: 53 - protein, 18 aa, Clostridium phytofermentans
DNADLVASITRKVMEQLG

SEQ ID NO: 54 - protein, 20 aa, Clostridium phytofermentans
VNEQLVQDIIKNVVASMQLT

SEQ ID NO: 55 - protein, 21 aa, Clostridium kluyveri
EPEDNEDVQAIVKAIMAKLNL

SEQ ID NO: 56 - protein, 19 aa, Planctomyces limnophilus
DTEMLVKMITEQVMAALKK

SEQ ID NO: 57 - protein, 20 aa, Planctomyces limnophilus
MQATEQAIRQVVQEVLAQLN

SEQ ID NO: 58 - protein, 18 aa, Opitutus terrae
EVEALVQRLTEEILRQLQ

SEQ ID NO: 59 - protein, 17 aa, Opitutus terrae
IDETLVRSVVEEVVRAF

SEQ ID NO: 60 - protein, 15 aa, Clostridium phytofermentans
EDARDLLKQILQALS

SEQ ID NO: 61 - protein, 17 aa, Clostridium phytofermentans
MDIREFSNKFVEATKNM

SEQ ID NO: 62 - protein, 22 aa, Mycobacterium smegmatis
LDALRAELRALVVEELAQLIKR

SEQ ID NO: 63 - protein, 19 aa, Haliangium ochraceum
MALREDRIAEIVERVLARL

SEQ ID NO: 64 - protein, 39 aa, Artificial sequence
  Synthetic Sequence
MEINEKLLRQIIEDVLSEPMGSSHHHHHHSSGLVPRGSH

SEQ ID NO: 65 - protein, 39 aa, Artificial Sequence
  Synthetic Sequence
MNTSELETLIRNILSEQLAMGSSHHHHHHSSGLVPRGSH

SEQ ID NO: 66 - DNA, 29 bp, Artificial Sequence
  Primer GldA_NdeI_FW
catcatatggaccgcattattcaatcacc

SEQ ID NO: 67 - DNA, 28 bp, Artificial Sequence
  Primer GldA_SpeI_RV
catactagtttattcccactcttgcagg

SEQ ID NO: 68 - DNA, 36 bp, Artificial Sequence
  Primer dhaK_NdeI_FW
cgccatatgtctcaattcttttttaaccaacgcacc

SEQ ID NO: 69 - DNA, 30 bp, Artificial Sequence
  Primer dhaK_SpeI_RV
catactagtttagcccagctcactctccgc

SEQ ID NO: 70 - DNA, 32 bp, Artificial Sequence
  Primer mgsA_NdeI_FW
catcatatggaactgacgactcgcactttacc

SEQ ID NO: 71 - DNA, 30 bp, Artificial Sequence
  Primer mgsA_SpeI_RV
catactagtttacttcagacggtccgcgag

SEQ ID NO: 72 - DNA, 27 bp, Artificial Sequence
  Primer fucO_NdeI_FW
ccgcatatggctaacagaatgattctg

SEQ ID NO: 73 - DNA, 25 bp, Artificial Sequence
  Primer fucO_SpeI_RV
cctactagtttaccaggcggtatgg

SEQ ID NO: 74 - DNA, 30 bp, Artificial Sequence
  Primer GFP_NdeI_FW
gtacatatgagcaaaggagaagaacttttc

SEQ ID NO: 75 - DNA, 66 bp, Artificial Sequence
  Primer GFP-SsrA_SpeI_RV
gacactagtttaagctgctaaagcgtagttttcgtcgtttgctgctttgtacagctcatccatgcc

SEQ ID NO: 76 - protein, 9 aa, Artificial Sequence
  Synthetic Sequence
  MISC_FEATURE (1)..(1): hydrophobic amino acid
  MISC_FEATURE (2)..(2): polar or charged amino acid
  MISC_FEATURE (3)..(3): polar or charged amino acid
  MISC_FEATURE (4)..(4): hydrophobic amino acid
  MISC_FEATURE (5)..(5): hydrophobic amino acid
  MISC_FEATURE (6)..(6): polar or charged amino acid
  MISC_FEATURE (7)..(7): any amino acid
  MISC_FEATURE (8)..(8): hydrophobic amino acid
  MISC_FEATURE (9)..(9): hydrophobic amino acid
XXXXXXXXX

SEQ ID NO: 77 - protein, 9 aa, Artificial Sequence
  Synthetic Sequence
  VARIANT (1)..(1): /replace="Leu" /replace="Val" /replace="Met" /replace="Phe" /replace="Tyr" /replace="Ala" /replace="Trp"
  VARIANT (2)..(2): /replace="Asn" /replace="Thr" /replace="Ser" /replace="Cys" /replace="Asp" /replace="Glu" /replace="Arg" /replace="Lys" /replace="His"
  VARIANT (3)..(3): /replace="Asn" /replace="Thr" /replace="Ser" /replace="Cys" /replace="Asp" /replace="Glu" /replace="Arg" /replace="Lys" /replace="His"
  VARIANT (4)..(4): /replace="Leu" /replace="Val" /replace="Met" /replace="Phe" /replace="Tyr" /replace="Ala" /replace="Trp"
  VARIANT (5)..(5): /replace="Leu" /replace="Val" /replace="Met" /replace="Phe" /replace="Tyr" /replace="Ala" /replace="Trp"
  VARIANT (6)..(6): /replace="Asn" /replace="Thr" /replace="Ser" /replace="Cys" /replace="Asp" /replace="Glu" /replace="Arg" /replace="Lys" /replace="His"
  MISC_FEATURE (7)..(7): any amino acid
  VARIANT (8)..(8): /replace="Leu" /replace="Val" /replace="Met" /replace="Phe" /replace="Tyr" /replace="Ala" /replace="Trp"
  VARIANT (9)..(9): /replace="Leu" /replace="Val" /replace="Met" /replace="Phe" /replace="Tyr" /replace="Ala" /replace="Trp"
IQQIIQXII

SEQ ID NO: 78 - protein, 9 aa, Artificial Sequence
  Synthetic Sequence
  VARIANT (1)..(1): /replace="Leu" /replace="Val" /replace="Met" /replace="Ala"
  VARIANT (2)..(2): /replace="Thr" /replace="Glu" /replace="Arg" /replace="Ser" /replace="Asp" /replace="Lys"
  VARIANT (3)..(3): /replace="Thr" /replace="Glu" /replace="Arg" /replace="Ser" /replace="Asp" /replace="Lys"
  VARIANT (4)..(4): /replace="Leu" /replace="Val" /replace="Met" /replace="Ala"
  VARIANT (5)..(5): /replace="Leu" /replace="Val" /replace="Met" /replace="Ala"
  VARIANT (6)..(6): /replace="Thr" /replace="Glu" /replace="Arg" /replace="Ser" /replace="Asp" /replace="Lys"
  MISC_FEATURE (7)..(7): any amino acid
  VARIANT (8)..(8): /replace="Leu" /replace="Val" /replace="Met" /replace="Ala"
  VARIANT (9)..(9): /replace="Leu" /replace="Val" /replace="Met" /replace="Ala"
IQQIIQXII

SEQ ID NO: 79 - protein, 9 aa, Artificial Sequence
  Artificial Sequence
  VARIANT (1)..(1): /replace="Leu" /replace="Val" /replace="Ala"
  VARIANT (2)..(2): /replace="Glu" /replace="Arg"
  VARIANT (3)..(3): /replace="Thr" /replace="Glu" /replace="Ser" /replace="Asp" /replace="Lys"
  VARIANT (4)..(4): /replace="Leu" /replace="Val" /replace="Met"
  VARIANT (5)..(5): /replace="Leu" /replace="Val"
  VARIANT (6)..(6): /replace="Arg" /replace="Lys" /replace="Glu"
  MISC_FEATURE (7)..(7): any amino acid
  VARIANT (8)..(8): /replace="Leu" /replace="Val" /replace="Ala"
  VARIANT (9)..(9): /replace="Leu" /replace="Val" /replace="Met"
IQQIIQXII